European Patent Specification EP 3 848 709 B1, published December 4, 2024. Title: Compositions and methods for detecting and treating esophageal cancer. Applicant: Progastrine et Cancers S.à r.l. The sequence listing filed with the application follows.

SEQUENCE LISTING (40 sequences)

SEQ ID NO: 1 - protein, 80 aa, Homo sapiens
  SITE (1)..(80): Human progastrin
SWKPRSQQPDAPLGTGANRDLELPWLEQQGPASHHRRQLGPQGPPHLVADPSKKQGPWLEEEEEAYGWMDFGRRSAEDEN

SEQ ID NO: 2 - protein, 14 aa, Artificial
  Amino acids 1-14, N-terminal extremity of human progastrin
SWKPRSQQPDAPLG

SEQ ID NO: 3 - protein, 26 aa, Artificial
  Amino acids 55-80, C-terminal extremity of human progastrin
QGPWLEEEEEAYGWMDFGRRSAEDEN

SEQ ID NO: 4 - protein, 8 aa, Artificial
  6B5B11C10 CDR-H1
GYIFTSYW

SEQ ID NO: 5 - protein, 8 aa, Artificial
  6B5B11C10 CDR-H2
FYPGNSDS

SEQ ID NO: 6 - protein, 8 aa, Artificial
  6B5B11C10 CDR-H3
TRRDSPQY

SEQ ID NO: 7 - protein, 11 aa, Artificial
  6B5B11C10 CDR-L1
QSIVHSNGNTY

SEQ ID NO: 8 - protein, 3 aa, Artificial
  6B5B11C10 CDR-L2
KVS

SEQ ID NO: 9 - protein, 9 aa, Artificial
  6B5B11C10 CDR-L3
FQGSHVPFT

SEQ ID NO: 10 - protein, 7 aa, Artificial
  20D2C3G2 CDR-H1
GYTFSSW

SEQ ID NO: 11 - protein, 8 aa, Artificial
  20D2C3G2 CDR-H2
FLPGSGST

SEQ ID NO: 12 - protein, 11 aa, Artificial
  20D2C3G2 CDR-H3
ATDGNYDWFAY

SEQ ID NO: 13 - protein, 11 aa, Artificial
  20D2C3G2 CDR-L1
QSLVHSSGVTY

SEQ ID NO: 14 - protein, 3 aa, Artificial
  20D2C3G2 CDR-L2
KVS

SEQ ID NO: 15 - protein, 9 aa, Artificial
  20D2C3G2 CDR-L3
SQSTHVPPT

SEQ ID NO: 16 - protein, 8 aa, Artificial
  1E9D9B6 CDR-H1
GYTFTSYY

SEQ ID NO: 17 - protein, 8 aa, Artificial
  1E9D9B6 CDR-H2
INPSNGGT

SEQ ID NO: 18 - protein, 10 aa, Artificial
  1E9D9B6 CDR-H3
TRGGYYPFDY

SEQ ID NO: 19 - protein, 11 aa, Artificial
  1E9D9B6 CDR-L1
QSLLDSDGKTY

SEQ ID NO: 20 - protein, 3 aa, Artificial
  1E9D9B6 CDR-L2
LVS

SEQ ID NO: 21 - protein, 9 aa, Artificial
  1E9D9B6 CDR-L3
WQGTHSPYT

SEQ ID NO: 22 - protein, 9 aa, Artificial
  1B3B4F11 CDR-H1
GYSITSDYA

SEQ ID NO: 23 - protein, 7 aa, Artificial
  1B3B4F11 CDR-H2
ISFSGYT

SEQ ID NO: 24 - protein, 14 aa, Artificial
  1B3B4F11 CDR-H3
AREVNYGDSYHFDY

SEQ ID NO: 25 - protein, 7 aa, Artificial
  1B3B4F11 CDR-L1
SQHRTYT

SEQ ID NO: 26 - protein, 7 aa, Artificial
  1B3B4F11 CDR-L2
VKKDGSH

SEQ ID NO: 27 - protein, 13 aa, Artificial
  1B3B4F11 CDR-L3
GVGDAIKGQSVFV

SEQ ID NO: 28 - protein, 8 aa, Artificial
  1C10D3B9 CDR-H1
GFTFTTYA

SEQ ID NO: 29 - protein, 8 aa, Artificial
  1C10D3B9 CDR-H2
ISSGGTYT

SEQ ID NO: 30 - protein, 10 aa, Artificial
  1C10D3B9 CDR-H3
ATQGNYSLDF

SEQ ID NO: 31 - protein, 11 aa, Artificial
  1C10D3B9 CDR-L1
KSLRHTKGITF

SEQ ID NO: 32 - protein, 3 aa, Artificial
  1C10D3B9 CDR-L2
QMS

SEQ ID NO: 33 - protein, 9 aa, Artificial
  1C10D3B9 CDR-L3
AQNLELPLT

SEQ ID NO: 34 - protein, 8 aa, Artificial
  2C6C3C7 CDR-H1
GFIFSSYG

SEQ ID NO: 35 - protein, 8 aa, Artificial
  2C6C3C7 CDR-H2
INTFGDRT

SEQ ID NO: 36 - protein, 7 aa, Artificial
  2C6C3C7 CDR-H3
ARGTGTY

SEQ ID NO: 37 - protein, 11 aa, Artificial
  2C6C3C7 CDR-L1
QSLLDSDGKTY

SEQ ID NO: 38 - protein, 3 aa, Artificial
  2C6C3C7 CDR-L2
LVS

SEQ ID NO: 39 - protein, 9 aa, Artificial
  2C6C3C7 CDR-L3
WQGTHFPQT

SEQ ID NO: 40 - protein, 10 aa, Artificial
  Amino acids 71-80 of progastrin
FGRRSAEDEN